European Patent Specification EP 4 008 347 B1, published April 30, 2025. Title: Antigen binding molecule. Applicant: MIE UNIVERSITY CHUBU UNIVERSITY EDUCATIONAL FOUNDATION. The sequence listing filed with the application follows.

SEQUENCE LISTING (41 sequences)

SEQ ID NO: 1 - protein, 8 aa, Artificial Sequence
  H CDR1
GFSLPSYG

SEQ ID NO: 2 - protein, 8 aa, Artificial Sequence
  H CDR2
IWAGGITN

SEQ ID NO: 3 - protein, 12 aa, Artificial Sequence
  H CDR3
ARGGSDYDGFAY

SEQ ID NO: 4 - protein, 117 aa, Artificial Sequence
  H variable region
EVQLVESGPGLVAPSQSLSITCTVSGFSLPSYGVHWVRQPPGKGLEWLGVIWAGGITNYNSALMSRLTISKDNSKSQVFLKMNSLQTDDTAIYYCARGGSDYDGFAYWGQGTLVTVS

SEQ ID NO: 5 - DNA, 24 bp, Artificial Sequence
  H CDR1
gggttttcattacccagctatggt

SEQ ID NO: 6 - DNA, 24 bp, Artificial Sequence
  H CDR2
atctgggctggtggaatcacaaat

SEQ ID NO: 7 - DNA, 36 bp, Artificial Sequence
  H CDR3
gccagaggcggctctgattacgacggctttgcttac

SEQ ID NO: 8 - DNA, 357 bp, Artificial Sequence
  H variable region
gaggtgcagctggtggagtctggacctggcctggtggcgccctcacagagcctgtccatcacttgcactgtctctgggttttcattacccagctatggtgttcactgggttcgccagcctccaggaaagggtctggagtggctgggagtaatctgggctggtggaatcacaaattataactcggctctcatgtccagactgaccatcagcaaagacaactccaagagccaagttttcttaaaaatgaacagtcttcaaactgatgacacagccatatactactgtgccagaggcggctctgattacgacggctttgcttactggggccaagggactctggtcactgtctctgcatca

SEQ ID NO: 9 - protein, 12 aa, Artificial Sequence
  L CDR1
QSLLSSRTRKNY

SEQ ID NO: 10 - protein, 3 aa, Artificial Sequence
  L CDR2
WAS

SEQ ID NO: 11 - protein, 8 aa, Artificial Sequence
  L CDR3
KQSYNLRT

SEQ ID NO: 12 - protein, 112 aa, Artificial Sequence
  L variable region
DIVMTQSPSSLAVSAGEKVTMNCRSSQSLLSSRTRKNYLAWYQQKPGQSPKLLIYWASIRESGVPDRFTGSGSGTDFTLTISSVQAEDLAVYYCKQSYNLRTFGGGTKLEIK

SEQ ID NO: 13 - DNA, 36 bp, Artificial Sequence
  L CDR1
cagagtctcctcagcagtagaacccgaaagaactac

SEQ ID NO: 14 - DNA, 9 bp, Artificial Sequence
  L CDR2
tgggcatct

SEQ ID NO: 15 - DNA, 24 bp, Artificial Sequence
  L CDR3
aagcaatcttataatcttcggacg

SEQ ID NO: 16 - DNA, 336 bp, Artificial Sequence
  L variable region
gacattgtgatgacacagtctccatcctccctggctgtgtcagcaggagagaaggtcactatgaactgcagatccagtcagagtctcctcagcagtagaacccgaaagaactacttggcttggtaccagcagaaaccagggcagtctcctaaactgctgatctactgggcatctattagggaatctggggtccctgatcgcttcacaggcagtggatctgggacagatttcactctcaccatcagcagtgtgcaggctgaagacctggcagtttattactgcaagcaatcttataatcttcggacgttcggtggaggcaccaagctggaaatcaaa

SEQ ID NO: 17 - DNA, 12 bp, Artificial Sequence
  NotI site kozak sequence
gcggccgccacc

SEQ ID NO: 18 - DNA, 57 bp, Artificial Sequence
  mVH leader
atgaactttgggctcagattgattttccttgtccttactttaaaaggtgtgaagtgt

SEQ ID NO: 19 - DNA, 357 bp, Artificial Sequence; identical to SEQ ID NO: 8
  mVH

SEQ ID NO: 20 - DNA, 45 bp, Artificial Sequence
  single chain
ggaggtggaggttctggtggaggaggttcaggtggaggtggatca

SEQ ID NO: 21 - DNA, 336 bp, Artificial Sequence; identical to SEQ ID NO: 16
  mVkappa

SEQ ID NO: 22 - DNA, 330 bp, Artificial Sequence
  hCkappa
cgaactgtggctgcaccatctgtcttcatcttcccgccatctgatgagcagttgaaatctggaactgcctctgttgtgtgcctgctgaataacttctatcccagagaggccaaagtacagtggaaggtggataacgccctccaatcgggtaactcccaggagagtgtcacagagcaggacagcaaggacagcacctacagcctcagcagcaccctgacgctgagcaaagcggactacgagaaacacaaactctacgcctgcgaagtcacccatcagggcctgagctcgcccgtcacaaagagcttcaacaggggagagtgtggcgcgcca

SEQ ID NO: 23 - DNA, 90 bp, Artificial Sequence
  hCD28 transmembrane
actagattttgggtgctggtggtggttggtggagtcctggcttgctatagcttgctagtaacagtggcctttattattttctgggtgagg

SEQ ID NO: 24 - DNA, 120 bp, Artificial Sequence
  hCD28 intracellular domain
agtaagaggagcaggctcctgcacagtgactacatgaacatgactccccgccgccccgggcccacccgcaagcattaccagccctatgccccaccacgcgacttcgcagcctatcgctcc

SEQ ID NO: 25 - DNA, 342 bp, Artificial Sequence
  hCD3 zeta
ctgagagtgaagttcagcaggagcgcagacgcccccgcgtaccagcagggccagaaccagctctataacgagctcaatctaggacgaagagaggagtacgatgttttggacaagagacgtggccgggaccctgagatggggggaaagccgcagagaaggaagaaccctcaggaaggcctgtacaatgaactgcagaaagataagatggcggaggcctacagtgagattgggatgaaaggcgagcgccggaggggcaaggggcacgatggcctttaccagggtctcagtacagccaccaaggacacctacgacgcccttcacatgcaggccctgccccctcgc

SEQ ID NO: 26 - DNA, 12 bp, Artificial Sequence
  XhoI site
tcgattctcgag

SEQ ID NO: 27 - protein, 19 aa, Artificial Sequence
  mVH leader
MNFGLRLIFLVLTLKGVKC

SEQ ID NO: 28 - protein, 117 aa, Artificial Sequence; identical to SEQ ID NO: 4
  mVH

SEQ ID NO: 29 - protein, 15 aa, Artificial Sequence
  single chain
GGGGSGGGGSGGGGS

SEQ ID NO: 30 - protein, 112 aa, Artificial Sequence; identical to SEQ ID NO: 12
  mVkappa

SEQ ID NO: 31 - protein, 110 aa, Artificial Sequence
  hCkappa
RTVAAPSVFIFPPSDEQLKSGTASVVCLLNNFYPREAKVQWKVDNALQSGNSQESVTEQDSKDSTYSLSSTLTLSKADYEKHKLYACEVTHQGLSSPVTKSFNRGECGAP

SEQ ID NO: 32 - protein, 30 aa, Artificial Sequence
  hCD28 transmembrane
TRFWVLVVVGGVLACYSLLVTVAFIIFWVR

SEQ ID NO: 33 - protein, 40 aa, Artificial Sequence
  hCD28 intracellular domain
SKRSRLLHSDYMNMTPRRPGPTRKHYQPYAPPRDFAAYRS

SEQ ID NO: 34 - protein, 114 aa, Artificial Sequence
  hCD3 zeta
LRVKFSRSADAPAYQQGQNQLYNELNLGRREEYDVLDKRRGRDPEMGGKPQRRKNPQEGLYNELQKDKMAEAYSEIGMKGERRRGKGHDGLYQGLSTATKDTYDALHMQALPPR

SEQ ID NO: 35 - DNA, 147 bp, Artificial Sequence
  hGITR intracellular domain
aggagtcagtgcatgtggccccgagagacccagctgctgctggaggtgccgccgtcgaccgaagacgccagaagctgccagttccccgaggaagagcggggcgagcgatcggcagaggagaaggggcggctgggagacctgtgggtg

SEQ ID NO: 36 - protein, 49 aa, Artificial Sequence
  hGITR intracellular domain
RSQCMWPRETQLLLEVPPSTEDARSCQFPEEERGERSAEEKGRLGDLWV

SEQ ID NO: 37 - DNA, 66 bp, Artificial Sequence
  P2A
ggatccggcgccacaaattttagcctcttgaagcaagccggcgacgtggaagagaatcctgggccc

SEQ ID NO: 38 - DNA, 597 bp, Artificial Sequence
  GITRL
atgaccctgcaccccagccccatcacctgcgagttcctgttcagcaccgccctgatcagccccaagatgtgcctgagccacctggagaacatgcccctgagccacagcagaacccagggcgcccagagaagcagctggaagctgtggctgttctgcagcatcgtgatgctgctgttcctgtgcagcttcagctggctgatcttcatcttcctgcagctggagaccgccaaggagccctgcatggccaagttcggccccctgcccagcaagtggcagatggccagcagcgagcccccctgcgtgaacaaggtgagcgactggaagctggagatcctgcagaacggcctgtacctgatctacggccaggtggcccccaacgccaactacaacgacgtggcccccttcgaggtgagactgtacaagaacaaggacatgatccagaccctgaccaacaagagcaagatccagaacgtgggcggcacctacgagctgcacgtgggcgacaccatcgacctgatcttcaacagcgagcaccaggtgctgaagaacaacacctactggggcatcatcctgctggccaacccccagttcatcagc

SEQ ID NO: 39 - protein, 22 aa, Artificial Sequence
  P2A
GSGATNFSLLKQAGDVEENPGP

SEQ ID NO: 40 - protein, 199 aa, Artificial Sequence
  GITRL
MTLHPSPITCEFLFSTALISPKMCLSHLENMPLSHSRTQGAQRSSWKLWLFCSIVMLLFLCSFSWLIFIFLQLETAKEPCMAKFGPLPSKWQMASSEPPCVNKVSDWKLEILQNGLYLIYGQVAPNANYNDVAPFEVRLYKNKDMIQTLTNKSKIQNVGGTYELHVGDTIDLIFNSEHQVLKNNTYWGIILLANPQFIS

SEQ ID NO: 41 - protein, 5 aa, Artificial Sequence
  GS linker
GGGGS